European Patent Application EP 4 703 389 A1, published March 4, 2026. Title: 抗PTK7抗体及其用途. Applicant: 上海麦科思生物医药有限公司. The sequence listing filed with the application follows.

SEQUENCE LISTING (27 sequences)

SEQ ID NO: 1 - protein, 5 aa, synthetic construct
DYGMH

SEQ ID NO: 2 - protein, 17 aa, synthetic construct
VISPYYGDVNYNQKFQG

SEQ ID NO: 3 - protein, 4 aa, synthetic construct
GMGY

SEQ ID NO: 4 - protein, 11 aa, synthetic construct
RASQSISKYLA

SEQ ID NO: 5 - protein, 7 aa, synthetic construct
SGSTLQS

SEQ ID NO: 6 - protein, 9 aa, synthetic construct
QQHNEYPWT

SEQ ID NO: 7 - protein, 7 aa, synthetic construct
GYTFTDY

SEQ ID NO: 8 - protein, 6 aa, synthetic construct
SPYYGD

SEQ ID NO: 9 - skipped

SEQ ID NO: 10 - protein, 11 aa, synthetic construct
RASQSISKYLA

SEQ ID NO: 11 - protein, 7 aa, synthetic construct
SGSTLQS

SEQ ID NO: 12 - protein, 9 aa, synthetic construct
QQHNEYPWT

SEQ ID NO: 13 - protein, 8 aa, synthetic construct
GYTFTDYG

SEQ ID NO: 14 - protein, 8 aa, synthetic construct
ISPYYGDV

SEQ ID NO: 15 - protein, 6 aa, synthetic construct
ARGMGY

SEQ ID NO: 16 - protein, 6 aa, synthetic construct
QSISKY

SEQ ID NO: 17 - skipped

SEQ ID NO: 18 - protein, 9 aa, synthetic construct
QQHNEYPWT

SEQ ID NO: 19 - protein, 107 aa, synthetic construct
DVQITQSPSYLAASPGETITINCRASQSISKYLAWYQEKPGKTNKLLIYSGSTLQSGIPSRFSGSGSGTDFTLTISSLEPEDFAMYYCQQHNEYPWTFGGGTKLEIK

SEQ ID NO: 20 - protein, 113 aa, synthetic construct
QVQLQQSGAELVRPGVSVKISCKGSGYTFTDYGMHWLKQSHAKSLEWIGVISPYYGDVTYNQKFKGKATMTVDKSSSTAYMELARLTSEDSAIYYCARGMGYWGQGTSVTVSS

SEQ ID NO: 21 - protein, 113 aa, synthetic construct
QVQLVQSGAEVKKPGASVKVSCKGSGYTFTDYGMHWLRQAPGQGLEWMGVISPYYGDVNYNQKFQGRVTMTRDKSISTAYMELSRLRSDDTVVYYCARGMGYWGQGTLVTVSS

SEQ ID NO: 22 - protein, 113 aa, synthetic construct
QVQLVQSGAEVKKPGASVKISCKGSGYTFTDYGMHWLKQAPGQGLEWIGVISPYYGDVNYNQKFQGRATMTVDKSISTAYMELSRLRSDDTAVYYCARGMGYWGQGTLVTVSS

SEQ ID NO: 23 - protein, 107 aa, synthetic construct
DIQLTQSPSFLSASVGDRVTITCRASQSISKYLAWYQQKPGKAPKLLIYSGSTLQSGVPSRFSGSGSGTEFTLTISSLQPEDFATYYCQQHNEYPWTFGQGTKVEIK

SEQ ID NO: 24 - protein, 107 aa, synthetic construct
DVQITQSPSFLSASVGDRVTITCRASQSISKYLAWYQQKPGKAPKLLIYSGSTLQSGVPSRFSGSGSGTEFTLTISSLQPEDFAMYYCQQHNEYPWTFGQGTKVEIK

SEQ ID NO: 25 - protein, 107 aa, synthetic construct
DVQITQSPSYLSASPGDRITITCRASQSISKYLAWYQQKPGKANKLLIYSGSTLQSGVPSRFSGSGSGTEFTLTISSLQPEDFAMYYCQQHNEYPWTFGQGTKVEIK

SEQ ID NO: 26 - protein, 448 aa, synthetic construct
QVQLVQSGPEVKKPGASVKVSCKASGYTFTDYAVHWVRQAPGKRLEWIGVISTYNDYTYNNQDFKGRVTMTRDTSASTAYMELSRLRSEDTAVYYCARGNSYFYALDYWGQGTSVTVSSASTKGPSVFPLAPSSKSTSGGTAALGCLVKDYFPEPVTVSWNSGALTSGVHTFPAVLQSSGLYSLSSVVTVPSSSLGTQTYICNVNHKPSNTKVDKKVEPKSCDKTHTCPPCPAPELLGGPSVFLFPPKPKDTLMISRTPEVTCVVVDVSHEDPEVKFNWYVDGVEVHNAKTKPREEQYNSTYRVVSVLTVLHQDWLNGKEYKCKVSNKALPAPIEKTISKAKGQPREPQVYTLPPSRDELTKNQVSLTCLVKGFYPSDIAVEWESNGQPENNYKTTPPVLDSDGSFFLYSKLTVDKSRWQQGNVFSCSVMHEALHNHYTQKSLSLSPG

SEQ ID NO: 27 - protein, 218 aa, synthetic construct
EIVLTQSPATLSLSPGERATLSCRASESVDSYGKSFMHWYQQKPGQAPRLLIYRASNLESGIPARFSGSGSGTDFTLTISSLEPEDFAVYYCQQSNEDPWTFGGGTKLEIKRTVAAPSVFIFPPSDEQLKSGTASVVCLLNNFYPREAKVQWKVDNALQSGNSQESVTEQDSKDSTYSLSSTLTLSKADYEKHKVYACEVTHQGLSSPVTKSFNRGEC